European Patent Specification EP 4 025 702 B1, published July 29, 2026. Title: ALPHA-SYNUCLEIN DETECTION USING BEADS. Applicant: Amprion, Inc. The sequence listing filed with the application follows.

SEQUENCE LISTING (19 sequences)

SEQ ID NO: 1 - protein, 140 aa, Artificial Sequence
  Synthetic
MDVFMKGLSKAKEGVVAAAEKTKQGVAEAAGKTKEGVLYVGSKTKEGVVHGVATVAEKTKEQVTNVGGAVVTGVTAVAQKTVEGAGSIAAATGFVKKDQLGKNEEGAPQEGILEDMPVDPDNEAYEMPSEEGYQDYEPEA

SEQ ID NO: 2 - protein, 146 aa, Artificial Sequence
  Synthetic
MDVFMKGLSKAKEGVVAAAEKTKQGVAEAAGKTKEGVLYVGSKTKEGVVHGVATVAEKTKEQVTNVGGAVVTGVTAVAQKTVEGAGSIAAATGFVKKDQLGKNEEGAPQEGILEDMPVDPDNEAYEMPSEEGYQDYEPEAHHHHHH

SEQ ID NO: 3 - protein, 146 aa, Artificial Sequence
  Synthetic
HHHHHHMDVFMKGLSKAKEGVVAAAEKTKQGVAEAAGKTKEGVLYVGSKTKEGVVHGVATVAEKTKEQVTNVGGAVVTGVTAVAQKTVEGAGSIAAATGFVKKDQLGKNEEGAPQEGILEDMPVDPDNEAYEMPSEEGYQDYEPEA

SEQ ID NO: 4 - protein, 147 aa, Artificial Sequence
  Synthetic
MDVFMKGLSKAKEGVVAAAEKTKQGVAEAAGKTKEGVLYVGSKTKEGVVHGVATVAEKTKEQVTNVGGAVVTGVTAVAQKTVEGAGSIAAATGFVKKDQLGKNEEGAPQEGILEDMPVDPDNEAYEMPSEEGYQDYEPEADYKDDDD

SEQ ID NO: 5 - protein, 147 aa, Artificial Sequence
  Synthetic
DYKDDDDMDVFMKGLSKAKEGVVAAAEKTKQGVAEAAGKTKEGVLYVGSKTKEGVVHGVATVAEKTKEQVTNVGGAVVTGVTAVAQKTVEGAGSIAAATGFVKKDQLGKNEEGAPQEGILEDMPVDPDNEAYEMPSEEGYQDYEPEA

SEQ ID NO: 6 - protein, 148 aa, Artificial Sequence
  Synthetic
MDVFMKGLSKAKEGVVAAAEKTKQGVAEAAGKTKEGVLYVGSKTKEGVVHGVATVAEKTKEQVTNVGGAVVTGVTAVAQKTVEGAGSIAAATGFVKKDQLGKNEEGAPQEGILEDMPVDPDNEAYEMPSEEGYQDYEPEADYKDDDDK

SEQ ID NO: 7 - protein, 148 aa, Artificial Sequence
  Synthetic
DYKDDDDKMDVFMKGLSKAKEGVVAAAEKTKQGVAEAAGKTKEGVLYVGSKTKEGVVHGVATVAEKTKEQVTNVGGAVVTGVTAVAQKTVEGAGSIAAATGFVKKDQLGKNEEGAPQEGILEDMPVDPDNEAYEMPSEEGYQDYEPEA

SEQ ID NO: 8 - protein, 147 aa, Artificial Sequence
  Synthetic
MDVFMKGLSKAKEGVVAAAEKTKQGVAEAAGKTKEGVLYVGSKTKEGVVHGVATVAEKTKEQVTNVGGAVVTGVTAVAQKTVEGAGSIAAATGFVKKDQLGKNEEGAPQEGILEDMPVDPDNEAYEMPSEEGYQDYEPEADYKDDDK

SEQ ID NO: 9 - protein, 147 aa, Artificial Sequence
  Synthetic
DYKDDDKMDVFMKGLSKAKEGVVAAAEKTKQGVAEAAGKTKEGVLYVGSKTKEGVVHGVATVAEKTKEQVTNVGGAVVTGVTAVAQKTVEGAGSIAAATGFVKKDQLGKNEEGAPQEGILEDMPVDPDNEAYEMPSEEGYQDYEPEA

SEQ ID NO: 10 - protein, 149 aa, Artificial Sequence
  Synthetic
MDVFMKGLSKAKEGVVAAAEKTKQGVAEAAGKTKEGVLYVGSKTKEGVVHGVATVAEKTKEQVTNVGGAVVTGVTAVAQKTVEGAGSIAAATGFVKKDQLGKNEEGAPQEGILEDMPVDPDNEAYEMPSEEGYQDYEPEAYPYDVPDYA

SEQ ID NO: 11 - protein, 149 aa, Artificial Sequence
  Synthetic
YPYDVPDYAMDVFMKGLSKAKEGVVAAAEKTKQGVAEAAGKTKEGVLYVGSKTKEGVVHGVATVAEKTKEQVTNVGGAVVTGVTAVAQKTVEGAGSIAAATGFVKKDQLGKNEEGAPQEGILEDMPVDPDNEAYEMPSEEGYQDYEPEA

SEQ ID NO: 12 - protein, 149 aa, Artificial Sequence
  Synthetic
MDVFMKGLSKAKEGVVAAAEKTKQGVAEAAGKTKEGVLYVGSKTKEGVVHGVATVAEKTKEQVTNVGGAVVTGVTAVAQKTVEGAGSIAAATGFVKKDQLGKNEEGAPQEGILEDMPVDPDNEAYEMPSEEGYQDYEPEAYAYDVPDYA

SEQ ID NO: 13 - protein, 149 aa, Artificial Sequence
  Synthetic
YAYDVPDYAMDVFMKGLSKAKEGVVAAAEKTKQGVAEAAGKTKEGVLYVGSKTKEGVVHGVATVAEKTKEQVTNVGGAVVTGVTAVAQKTVEGAGSIAAATGFVKKDQLGKNEEGAPQEGILEDMPVDPDNEAYEMPSEEGYQDYEPEA

SEQ ID NO: 14 - protein, 149 aa, Artificial Sequence
  Synthetic
MDVFMKGLSKAKEGVVAAAEKTKQGVAEAAGKTKEGVLYVGSKTKEGVVHGVATVAEKTKEQVTNVGGAVVTGVTAVAQKTVEGAGSIAAATGFVKKDQLGKNEEGAPQEGILEDMPVDPDNEAYEMPSEEGYQDYEPEAYDVPDYASL

SEQ ID NO: 15 - protein, 149 aa, Artificial Sequence
  Synthetic
YDVPDYASLMDVFMKGLSKAKEGVVAAAEKTKQGVAEAAGKTKEGVLYVGSKTKEGVVHGVATVAEKTKEQVTNVGGAVVTGVTAVAQKTVEGAGSIAAATGFVKKDQLGKNEEGAPQEGILEDMPVDPDNEAYEMPSEEGYQDYEPEA

SEQ ID NO: 16 - protein, 150 aa, Artificial Sequence
  Synthetic
MDVFMKGLSKAKEGVVAAAEKTKQGVAEAAGKTKEGVLYVGSKTKEGVVHGVATVAEKTKEQVTNVGGAVVTGVTAVAQKTVEGAGSIAAATGFVKKDQLGKNEEGAPQEGILEDMPVDPDNEAYEMPSEEGYQDYEPEAEQKLISEEDL

SEQ ID NO: 17 - protein, 150 aa, Artificial Sequence
  Synthetic
EQKLISEEDLMDVFMKGLSKAKEGVVAAAEKTKQGVAEAAGKTKEGVLYVGSKTKEGVVHGVATVAEKTKEQVTNVGGAVVTGVTAVAQKTVEGAGSIAAATGFVKKDQLGKNEEGAPQEGILEDMPVDPDNEAYEMPSEEGYQDYEPEA

SEQ ID NO: 18 - protein, 154 aa, Artificial Sequence
  Synthetic
MDVFMKGLSKAKEGVVAAAEKTKQGVAEAAGKTKEGVLYVGSKTKEGVVHGVATVAEKTKEQVTNVGGAVVTGVTAVAQKTVEGAGSIAAATGFVKKDQLGKNEEGAPQEGILEDMPVDPDNEAYEMPSEEGYQDYEPEAGKPIPNPLLGLDST

SEQ ID NO: 19 - protein, 154 aa, Artificial Sequence
  Synthetic
GKPIPNPLLGLDSTMDVFMKGLSKAKEGVVAAAEKTKQGVAEAAGKTKEGVLYVGSKTKEGVVHGVATVAEKTKEQVTNVGGAVVTGVTAVAQKTVEGAGSIAAATGFVKKDQLGKNEEGAPQEGILEDMPVDPDNEAYEMPSEEGYQDYEPEA